European Patent Application EP 4 471 051 A1, published December 4, 2024. Title: B DOMAIN AND Z DOMAIN MUTANTS OF PROTEIN A, AND APPLICATION THEREOF. Applicant: Bestchrom (Zhejiang) Biosciences Ltd. The sequence listing filed with the application follows.

SEQUENCE LISTING (124 sequences)

SEQ ID NO: 1 - protein, 58 aa, synthetic construct [sequence omitted]

SEQ ID NO: 2 - protein, 58 aa, synthetic construct [sequence omitted]

SEQ ID NO: 3 - protein, 58 aa, synthetic construct
VDLKFNKEQQNAFYEILHLPNLNEEQRNAFIQSLKDDPSQSANLLAEAKKLNDAQAPK

SEQ ID NO: 4 - protein, 58 aa, synthetic construct
VDVKFNKEQQNAFYEILHLPNLNEEQRNAFIQSLKDDPSQSANLLAEAKKLNDAQAPK

SEQ ID NO: 5 - protein, 58 aa, synthetic construct
VDYKFNKEQQNAFYEILHLPNLNEEQRNAFIQSLKDDPSQSANLLAEAKKLNDAQAPK

SEQ ID NO: 6 - protein, 58 aa, synthetic construct
VDNKFSKEQQNAFYEILHLPNLNEEQRNAFIQSLKDDPSQSANLLAEAKKLNDAQAPK

SEQ ID NO: 7 - protein, 58 aa, synthetic construct
VDNKFLKEQQNAFYEILHLPNLNEEQRNAFIQSLKDDPSQSANLLAEAKKLNDAQAPK

SEQ ID NO: 8 - protein, 58 aa, synthetic construct
VDNKFEKEQQNAFYEILHLPNLNEEQRNAFIQSLKDDPSQSANLLAEAKKLNDAQAPK

SEQ ID NO: 9 - protein, 58 aa, synthetic construct
VDNKFNKEIQNAFYEILHLPNLNEEQRNAFIQSLKDDPSQSANLLAEAKKLNDAQAPK

SEQ ID NO: 10 - protein, 58 aa, synthetic construct
VDNKFNKEFQNAFYEILHLPNLNEEQRNAFIQSLKDDPSQSANLLAEAKKLNDAQAPK

SEQ ID NO: 11 - protein, 58 aa, synthetic construct
VDNKFNKEMQNAFYEILHLPNLNEEQRNAFIQSLKDDPSQSANLLAEAKKLNDAQAPK

SEQ ID NO: 12 - protein, 58 aa, synthetic construct
VDNKFNKEQQNAFYTILHLPNLNEEQRNAFIQSLKDDPSQSANLLAEAKKLNDAQAPK

SEQ ID NO: 13 - protein, 58 aa, synthetic construct
VDNKFNKEQQNAFYWILHLPNLNEEQRNAFIQSLKDDPSQSANLLAEAKKLNDAQAPK

SEQ ID NO: 14 - protein, 58 aa, synthetic construct
VDNKFNKEQQNAFYLILHLPNLNEEQRNAFIQSLKDDPSQSANLLAEAKKLNDAQAPK

SEQ ID NO: 15 - protein, 58 aa, synthetic construct
VDNKFNKEQQNAFYVILHLPNLNEEQRNAFIQSLKDDPSQSANLLAEAKKLNDAQAPK

SEQ ID NO: 16 - protein, 58 aa, synthetic construct
VDNKFNKEQQNAFYIILHLPNLNEEQRNAFIQSLKDDPSQSANLLAEAKKLNDAQAPK

SEQ ID NO: 17 - protein, 58 aa, synthetic construct
VDNKFNKEQQNAFYFILHLPNLNEEQRNAFIQSLKDDPSQSANLLAEAKKLNDAQAPK

SEQ ID NO: 18 - protein, 58 aa, synthetic construct
VDNKFNKEQQNAFYSILHLPNLNEEQRNAFIQSLKDDPSQSANLLAEAKKLNDAQAPK

SEQ ID NO: 19 - protein, 58 aa, synthetic construct
VDNKFNKEQQNAFYYILHLPNLNEEQRNAFIQSLKDDPSQSANLLAEAKKLNDAQAPK

SEQ ID NO: 20 - protein, 58 aa, synthetic construct
VDNKFNKEQQNAFYDILHLPNLNEEQRNAFIQSLKDDPSQSANLLAEAKKLNDAQAPK

SEQ ID NO: 21 - protein, 58 aa, synthetic construct
VDNKFNKEQQNAFYEILHLPNLVEEQRNAFIQSLKDDPSQSANLLAEAKKLNDAQAPK

SEQ ID NO: 22 - protein, 58 aa, synthetic construct
VDNKFNKEQQNAFYEILHLPNLIEEQRNAFIQSLKDDPSQSANLLAEAKKLNDAQAPK

SEQ ID NO: 23 - protein, 58 aa, synthetic construct
VDNKFNKEQQNAFYEILHLPNLYEEQRNAFIQSLKDDPSQSANLLAEAKKLNDAQAPK

SEQ ID NO: 24 - protein, 58 aa, synthetic construct
VDNKFNKEIQNAFYTILHLPNLNEEQRNAFIQSLKDDPSQSANLLAEAKKLNDAQAPK

SEQ ID NO: 25 - protein, 58 aa, synthetic construct
VDNKFNKEIQNAFYWILHLPNLNEEQRNAFIQSLKDDPSQSANLLAEAKKLNDAQAPK

SEQ ID NO: 26 - protein, 58 aa, synthetic construct
VDNKFNKEIQNAFYLILHLPNLNEEQRNAFIQSLKDDPSQSANLLAEAKKLNDAQAPK

SEQ ID NO: 27 - protein, 58 aa, synthetic construct
VDNKFNKEIQNAFYVILHLPNLNEEQRNAFIQSLKDDPSQSANLLAEAKKLNDAQAPK

SEQ ID NO: 28 - protein, 58 aa, synthetic construct
VDNKFNKEIQNAFYIILHLPNLNEEQRNAFIQSLKDDPSQSANLLAEAKKLNDAQAPK

SEQ ID NO: 29 - protein, 58 aa, synthetic construct
VDNKFNKEIQNAFYFILHLPNLNEEQRNAFIQSLKDDPSQSANLLAEAKKLNDAQAPK

SEQ ID NO: 30 - protein, 58 aa, synthetic construct
VDNKFNKEIQNAFYSILHLPNLNEEQRNAFIQSLKDDPSQSANLLAEAKKLNDAQAPK

SEQ ID NO: 31 - protein, 58 aa, synthetic construct
VDNKFNKEIQNAFYYILHLPNLNEEQRNAFIQSLKDDPSQSANLLAEAKKLNDAQAPK

SEQ ID NO: 32 - protein, 58 aa, synthetic construct
VDNKFNKEIQNAFYDILHLPNLNEEQRNAFIQSLKDDPSQSANLLAEAKKLNDAQAPK

SEQ ID NO: 33 - protein, 58 aa, synthetic construct
VDNKFNKEFQNAFYTILHLPNLNEEQRNAFIQSLKDDPSQSANLLAEAKKLNDAQAPK

SEQ ID NO: 34 - protein, 58 aa, synthetic construct
VDNKFNKEFQNAFYWILHLPNLNEEQRNAFIQSLKDDPSQSANLLAEAKKLNDAQAPK

SEQ ID NO: 35 - protein, 58 aa, synthetic construct
VDNKFNKEFQNAFYLILHLPNLNEEQRNAFIQSLKDDPSQSANLLAEAKKLNDAQAPK

SEQ ID NO: 36 - protein, 58 aa, synthetic construct
VDNKFNKEFQNAFYVILHLPNLNEEQRNAFIQSLKDDPSQSANLLAEAKKLNDAQAPK

SEQ ID NO: 37 - protein, 58 aa, synthetic construct
VDNKFNKEFQNAFYIILHLPNLNEEQRNAFIQSLKDDPSQSANLLAEAKKLNDAQAPK

SEQ ID NO: 38 - protein, 58 aa, synthetic construct
VDNKFNKEFQNAFYFILHLPNLNEEQRNAFIQSLKDDPSQSANLLAEAKKLNDAQAPK

SEQ ID NO: 39 - protein, 58 aa, synthetic construct
VDNKFNKEFQNAFYSILHLPNLNEEQRNAFIQSLKDDPSQSANLLAEAKKLNDAQAPK

SEQ ID NO: 40 - protein, 58 aa, synthetic construct
VDNKFNKEFQNAFYYILHLPNLNEEQRNAFIQSLKDDPSQSANLLAEAKKLNDAQAPK

SEQ ID NO: 41 - protein, 58 aa, synthetic construct
VDNKFNKEFQNAFYDILHLPNLNEEQRNAFIQSLKDDPSQSANLLAEAKKLNDAQAPK

SEQ ID NO: 42 - protein, 58 aa, synthetic construct
VDLKFNKEIQNAFYLILHLPNLNEEQRNAFIQSLKDDPSQSANLLAEAKKLNDAQAPK

SEQ ID NO: 43 - protein, 58 aa, synthetic construct
VDYKFNKEIQNAFYVILHLPNLNEEQRNAFIQSLKDDPSQSANLLAEAKKLNDAQAPK

SEQ ID NO: 44 - protein, 58 aa, synthetic construct
VDVKFNKEIQNAFYIILHLPNLNEEQRNAFIQSLKDDPSQSANLLAEAKKLNDAQAPK

SEQ ID NO: 45 - protein, 58 aa, synthetic construct
VDNKFEKEIQNAFYLILHLPNLNEEQRNAFIQSLKDDPSQSANLLAEAKKLNDAQAPK

SEQ ID NO: 46 - protein, 58 aa, synthetic construct
VDNKFEKEFQNAFYVILHLPNLNEEQRNAFIQSLKDDPSQSANLLAEAKKLNDAQAPK

SEQ ID NO: 47 - protein, 58 aa, synthetic construct
VDNKFEKEIQNAFYIILHLPNLNEEQRNAFIQSLKDDPSQSANLLAEAKKLNDAQAPK

SEQ ID NO: 48 - protein, 58 aa, synthetic construct
VDVKFNKEIQNAFYLILHLPNLNEEQRNAFIQSLKDDPSQSANLLAEAKKLNDAQAPK

SEQ ID NO: 49 - protein, 58 aa, synthetic construct
VDVKFNKEIQNAFYVILHLPNLNEEQRNAFIQSLKDDPSQSANLLAEAKKLNDAQAPK

SEQ ID NO: 50 - protein, 58 aa, synthetic construct; identical to SEQ ID NO: 44

SEQ ID NO: 51 - protein, 58 aa, synthetic construct
VDLKFLKEIQNAFYLILHLPNLNEEQRNAFIQSLKDDPSQSANLLAEAKKLNDAQAPK

SEQ ID NO: 52 - protein, 58 aa, synthetic construct
VDYKFEKEIQNAFYIILHLPNLNEEQRNAFIQSLKDDPSQSANLLAEAKKLNDAQAPK

SEQ ID NO: 53 - protein, 58 aa, synthetic construct
VDVKFEKEIQNAFYLILHLPNLNEEQRNAFIQSLKDDPSQSANLLAEAKKLNDAQAPK

SEQ ID NO: 54 - protein, 58 aa, synthetic construct
VDLKFLKEFQNAFYIILHLPNLNEEQRNAFIQSLKDDPSQSANLLAEAKKLNDAQAPK

SEQ ID NO: 55 - protein, 58 aa, synthetic construct
VDYKFEKEIQNAFYLILHLPNLNEEQRNAFIQSLKDDPSQSANLLAEAKKLNDAQAPK

SEQ ID NO: 56 - protein, 58 aa, synthetic construct
VDVKFEKEIQNAFYIILHLPNLNEEQRNAFIQSLKDDPSQSANLLAEAKKLNDAQAPK

SEQ ID NO: 57 - protein, 58 aa, synthetic construct
VDLKFNKEIQNAFYLILHLPNLVEEQRNAFIQSLKDDPSQSANLLAEAKKLNDAQAPK

SEQ ID NO: 58 - protein, 58 aa, synthetic construct
VDYKFNKEIQNAFYIILHLPNLVEEQRNAFIQSLKDDPSQSANLLAEAKKLNDAQAPK

SEQ ID NO: 59 - protein, 58 aa, synthetic construct
VDVKFNKEIQNAFYLILHLPNLYEEQRNAFIQSLKDDPSQSANLLAEAKKLNDAQAPK

SEQ ID NO: 60 - protein, 58 aa, synthetic construct
VDNKFLKEFQNAFYIILHLPNLVEEQRNAFIQSLKDDPSQSANLLAEAKKLNDAQAPK

SEQ ID NO: 61 - protein, 58 aa, synthetic construct
VDNKFEKEIQNAFYLILHLPNLIEEQRNAFIQSLKDDPSQSANLLAEAKKLNDAQAPK

SEQ ID NO: 62 - protein, 58 aa, synthetic construct
VDNKFEKEIQNAFYLILHLPNLYEEQRNAFIQSLKDDPSQSANLLAEAKKLNDAQAPK

SEQ ID NO: 63 - protein, 58 aa, synthetic construct
VDLKFLKEIQNAFYLILHLPNLVEEQRNAFIQSLKDDPSQSANLLAEAKKLNDAQAPK

SEQ ID NO: 64 - protein, 58 aa, synthetic construct
VDLKFEKEIQNAFYIILHLPNLIEEQRNAFIQSLKDDPSQSANLLAEAKKLNDAQAPK

SEQ ID NO: 65 - protein, 58 aa, synthetic construct
VDVKFEKEIQNAFYLILHLPNLYEEQRNAFIQSLKDDPSQSANLLAEAKKLNDAQAPK

SEQ ID NO: 66 - protein, 58 aa, synthetic construct
VDVKFEKEIQNAFYIILHLPNLYEEQRNAFIQSLKDDPSQSANLLAEAKKLNDAQAPK

SEQ ID NO: 67 - protein, 58 aa, synthetic construct
VDYKFEKEIQNAFYLILHLPNLYEEQRNAFIQSLKDDPSQSANLLAEAKKLNDAQAPK

SEQ ID NO: 68 - protein, 58 aa, synthetic construct
VDVKFLKEIQNAFYVILHLPNLYEEQRNAFIQSLKDDPSQSANLLAEAKKLNDAQAPK

SEQ ID NO: 69 - protein, 58 aa, synthetic construct
VDLKFLKEFQNAFYIILHLPNLVEEQRNAFIQSLKDDPSQSANLLAEAKKLNDAQAPK

SEQ ID NO: 70 - protein, 58 aa, synthetic construct
VDLKFEKEFQNAFYLILHLPNLIEEQRNAFIQSLKDDPSQSANLLAEAKKLNDAQAPK

SEQ ID NO: 71 - protein, 58 aa, synthetic construct
VDVKFLKEFQNAFYVILHLPNLYEEQRNAFIQSLKDDPSQSANLLAEAKKLNDAQAPK

SEQ ID NO: 72 - protein, 232 aa, synthetic construct
VDNKFNKEQQNAFYEILHLPNLNEEQRNAFIQSLKDDPSQSANLLAEAKKLNDAQAPKVDNKFNKEQQNAFYEILHLPNLNEEQRNAFIQSLKDDPSQSANLLAEAKKLNDAQAPKVDNKFNKEQQNAFYEILHLPNLNEEQRNAFIQSLKDDPSQSANLLAEAKKLNDAQAPKVDNKFNKEQQNAFYEILHLPNLNEEQRNAFIQSLKDDPSQSANLLAEAKKLNDAQAPK

SEQ ID NO: 73 - protein, 232 aa, synthetic construct
VDLKFNKEQQNAFYEILHLPNLNEEQRNAFIQSLKDDPSQSANLLAEAKKLNDAQAPKVDLKFNKEQQNAFYEILHLPNLNEEQRNAFIQSLKDDPSQSANLLAEAKKLNDAQAPKVDLKFNKEQQNAFYEILHLPNLNEEQRNAFIQSLKDDPSQSANLLAEAKKLNDAQAPKVDLKFNKEQQNAFYEILHLPNLNEEQRNAFIQSLKDDPSQSANLLAEAKKLNDAQAPK

SEQ ID NO: 74 - protein, 232 aa, synthetic construct
VDVKFNKEQQNAFYEILHLPNLNEEQRNAFIQSLKDDPSQSANLLAEAKKLNDAQAPKVDVKFNKEQQNAFYEILHLPNLNEEQRNAFIQSLKDDPSQSANLLAEAKKLNDAQAPKVDVKFNKEQQNAFYEILHLPNLNEEQRNAFIQSLKDDPSQSANLLAEAKKLNDAQAPKVDVKFNKEQQNAFYEILHLPNLNEEQRNAFIQSLKDDPSQSANLLAEAKKLNDAQAPK

SEQ ID NO: 75 - protein, 232 aa, synthetic construct
VDNKFLKEQQNAFYEILHLPNLNEEQRNAFIQSLKDDPSQSANLLAEAKKLNDAQAPKVDNKFLKEQQNAFYEILHLPNLNEEQRNAFIQSLKDDPSQSANLLAEAKKLNDAQAPKVDNKFLKEQQNAFYEILHLPNLNEEQRNAFIQSLKDDPSQSANLLAEAKKLNDAQAPKVDNKFLKEQQNAFYEILHLPNLNEEQRNAFIQSLKDDPSQSANLLAEAKKLNDAQAPK

SEQ ID NO: 76 - protein, 232 aa, synthetic construct
VDNKFEKEQQNAFYEILHLPNLNEEQRNAFIQSLKDDPSQSANLLAEAKKLNDAQAPKVDNKFEKEQQNAFYEILHLPNLNEEQRNAFIQSLKDDPSQSANLLAEAKKLNDAQAPKVDNKFEKEQQNAFYEILHLPNLNEEQRNAFIQSLKDDPSQSANLLAEAKKLNDAQAPKVDNKFEKEQQNAFYEILHLPNLNEEQRNAFIQSLKDDPSQSANLLAEAKKLNDAQAPK

SEQ ID NO: 77 - protein, 232 aa, synthetic construct
VDNKFNKEIQNAFYEILHLPNLNEEQRNAFIQSLKDDPSQSANLLAEAKKLNDAQAPKVDNKFNKEIQNAFYEILHLPNLNEEQRNAFIQSLKDDPSQSANLLAEAKKLNDAQAPKVDNKFNKEIQNAFYEILHLPNLNEEQRNAFIQSLKDDPSQSANLLAEAKKLNDAQAPKVDNKFNKEIQNAFYEILHLPNLNEEQRNAFIQSLKDDPSQSANLLAEAKKLNDAQAPK

SEQ ID NO: 78 - protein, 232 aa, synthetic construct
VDNKFNKEFQNAFYEILHLPNLNEEQRNAFIQSLKDDPSQSANLLAEAKKLNDAQAPKVDNKFNKEFQNAFYEILHLPNLNEEQRNAFIQSLKDDPSQSANLLAEAKKLNDAQAPKVDNKFNKEFQNAFYEILHLPNLNEEQRNAFIQSLKDDPSQSANLLAEAKKLNDAQAPKVDNKFNKEFQNAFYEILHLPNLNEEQRNAFIQSLKDDPSQSANLLAEAKKLNDAQAPK

SEQ ID NO: 79 - protein, 232 aa, synthetic construct
VDNKFNKEMQNAFYEILHLPNLNEEQRNAFIQSLKDDPSQSANLLAEAKKLNDAQAPKVDNKFNKEMQNAFYEILHLPNLNEEQRNAFIQSLKDDPSQSANLLAEAKKLNDAQAPKVDNKFNKEMQNAFYEILHLPNLNEEQRNAFIQSLKDDPSQSANLLAEAKKLNDAQAPKVDNKFNKEMQNAFYEILHLPNLNEEQRNAFIQSLKDDPSQSANLLAEAKKLNDAQAPK

SEQ ID NO: 80 - protein, 232 aa, synthetic construct
VDNKFNKEQQNAFYTILHLPNLNEEQRNAFIQSLKDDPSQSANLLAEAKKLNDAQAPKVDNKFNKEQQNAFYTILHLPNLNEEQRNAFIQSLKDDPSQSANLLAEAKKLNDAQAPKVDNKFNKEQQNAFYTILHLPNLNEEQRNAFIQSLKDDPSQSANLLAEAKKLNDAQAPKVDNKFNKEQQNAFYTILHLPNLNEEQRNAFIQSLKDDPSQSANLLAEAKKLNDAQAPK

SEQ ID NO: 81 - protein, 232 aa, synthetic construct
VDNKFNKEQQNAFYWILHLPNLNEEQRNAFIQSLKDDPSQSANLLAEAKKLNDAQAPKVDNKFNKEQQNAFYWILHLPNLNEEQRNAFIQSLKDDPSQSANLLAEAKKLNDAQAPKVDNKFNKEQQNAFYWILHLPNLNEEQRNAFIQSLKDDPSQSANLLAEAKKLNDAQAPKVDNKFNKEQQNAFYWILHLPNLNEEQRNAFIQSLKDDPSQSANLLAEAKKLNDAQAPK

SEQ ID NO: 82 - protein, 232 aa, synthetic construct
VDNKFNKEQQNAFYLILHLPNLNEEQRNAFIQSLKDDPSQSANLLAEAKKLNDAQAPKVDNKFNKEQQNAFYLILHLPNLNEEQRNAFIQSLKDDPSQSANLLAEAKKLNDAQAPKVDNKFNKEQQNAFYLILHLPNLNEEQRNAFIQSLKDDPSQSANLLAEAKKLNDAQAPKVDNKFNKEQQNAFYLILHLPNLNEEQRNAFIQSLKDDPSQSANLLAEAKKLNDAQAPK

SEQ ID NO: 83 - protein, 232 aa, synthetic construct
VDNKFNKEQQNAFYVILHLPNLNEEQRNAFIQSLKDDPSQSANLLAEAKKLNDAQAPKVDNKFNKEQQNAFYVILHLPNLNEEQRNAFIQSLKDDPSQSANLLAEAKKLNDAQAPKVDNKFNKEQQNAFYVILHLPNLNEEQRNAFIQSLKDDPSQSANLLAEAKKLNDAQAPKVDNKFNKEQQNAFYVILHLPNLNEEQRNAFIQSLKDDPSQSANLLAEAKKLNDAQAPK

SEQ ID NO: 84 - protein, 232 aa, synthetic construct
VDNKFNKEQQNAFYIILHLPNLNEEQRNAFIQSLKDDPSQSANLLAEAKKLNDAQAPKVDNKFNKEQQNAFYIILHLPNLNEEQRNAFIQSLKDDPSQSANLLAEAKKLNDAQAPKVDNKFNKEQQNAFYIILHLPNLNEEQRNAFIQSLKDDPSQSANLLAEAKKLNDAQAPKVDNKFNKEQQNAFYIILHLPNLNEEQRNAFIQSLKDDPSQSANLLAEAKKLNDAQAPK

SEQ ID NO: 85 - protein, 232 aa, synthetic construct
VDNKFNKEQQNAFYFILHLPNLNEEQRNAFIQSLKDDPSQSANLLAEAKKLNDAQAPKVDNKFNKEQQNAFYFILHLPNLNEEQRNAFIQSLKDDPSQSANLLAEAKKLNDAQAPKVDNKFNKEQQNAFYFILHLPNLNEEQRNAFIQSLKDDPSQSANLLAEAKKLNDAQAPKVDNKFNKEQQNAFYFILHLPNLNEEQRNAFIQSLKDDPSQSANLLAEAKKLNDAQAPK

SEQ ID NO: 86 - protein, 232 aa, synthetic construct
VDNKFNKEQQNAFYSILHLPNLNEEQRNAFIQSLKDDPSQSANLLAEAKKLNDAQAPKVDNKFNKEQQNAFYSILHLPNLNEEQRNAFIQSLKDDPSQSANLLAEAKKLNDAQAPKVDNKFNKEQQNAFYSILHLPNLNEEQRNAFIQSLKDDPSQSANLLAEAKKLNDAQAPKVDNKFNKEQQNAFYSILHLPNLNEEQRNAFIQSLKDDPSQSANLLAEAKKLNDAQAPK

SEQ ID NO: 87 - protein, 232 aa, synthetic construct
VDNKFNKEQQNAFYYILHLPNLNEEQRNAFIQSLKDDPSQSANLLAEAKKLNDAQAPKVDNKFNKEQQNAFYYILHLPNLNEEQRNAFIQSLKDDPSQSANLLAEAKKLNDAQAPKVDNKFNKEQQNAFYYILHLPNLNEEQRNAFIQSLKDDPSQSANLLAEAKKLNDAQAPKVDNKFNKEQQNAFYYILHLPNLNEEQRNAFIQSLKDDPSQSANLLAEAKKLNDAQAPK

SEQ ID NO: 88 - protein, 232 aa, synthetic construct
VDNKFNKEQQNAFYDILHLPNLNEEQRNAFIQSLKDDPSQSANLLAEAKKLNDAQAPKVDNKFNKEQQNAFYDILHLPNLNEEQRNAFIQSLKDDPSQSANLLAEAKKLNDAQAPKVDNKFNKEQQNAFYDILHLPNLNEEQRNAFIQSLKDDPSQSANLLAEAKKLNDAQAPKVDNKFNKEQQNAFYDILHLPNLNEEQRNAFIQSLKDDPSQSANLLAEAKKLNDAQAPK

SEQ ID NO: 89 - protein, 232 aa, synthetic construct
VDNKFNKEQQNAFYEILHLPNLVEEQRNAFIQSLKDDPSQSANLLAEAKKLNDAQAPKVDNKFNKEQQNAFYEILHLPNLVEEQRNAFIQSLKDDPSQSANLLAEAKKLNDAQAPKVDNKFNKEQQNAFYEILHLPNLVEEQRNAFIQSLKDDPSQSANLLAEAKKLNDAQAPKVDNKFNKEQQNAFYEILHLPNLVEEQRNAFIQSLKDDPSQSANLLAEAKKLNDAQAPK

SEQ ID NO: 90 - protein, 232 aa, synthetic construct
VDNKFNKEQQNAFYEILHLPNLIEEQRNAFIQSLKDDPSQSANLLAEAKKLNDAQAPKVDNKFNKEQQNAFYEILHLPNLIEEQRNAFIQSLKDDPSQSANLLAEAKKLNDAQAPKVDNKFNKEQQNAFYEILHLPNLIEEQRNAFIQSLKDDPSQSANLLAEAKKLNDAQAPKVDNKFNKEQQNAFYEILHLPNLIEEQRNAFIQSLKDDPSQSANLLAEAKKLNDAQAPK

SEQ ID NO: 91 - protein, 232 aa, synthetic construct
VDNKFNKEQQNAFYEILHLPNLYEEQRNAFIQSLKDDPSQSANLLAEAKKLNDAQAPKVDNKFNKEQQNAFYEILHLPNLYEEQRNAFIQSLKDDPSQSANLLAEAKKLNDAQAPKVDNKFNKEQQNAFYEILHLPNLYEEQRNAFIQSLKDDPSQSANLLAEAKKLNDAQAPKVDNKFNKEQQNAFYEILHLPNLYEEQRNAFIQSLKDDPSQSANLLAEAKKLNDAQAPK

SEQ ID NO: 92 - protein, 232 aa, synthetic construct
VDNKFNKEIQNAFYLILHLPNLNEEQRNAFIQSLKDDPSQSANLLAEAKKLNDAQAPKVDNKFNKEIQNAFYLILHLPNLNEEQRNAFIQSLKDDPSQSANLLAEAKKLNDAQAPKVDNKFNKEIQNAFYLILHLPNLNEEQRNAFIQSLKDDPSQSANLLAEAKKLNDAQAPKVDNKFNKEIQNAFYLILHLPNLNEEQRNAFIQSLKDDPSQSANLLAEAKKLNDAQAPK

SEQ ID NO: 93 - protein, 232 aa, synthetic construct
VDNKFNKEIQNAFYVILHLPNLNEEQRNAFIQSLKDDPSQSANLLAEAKKLNDAQAPKVDNKFNKEIQNAFYVILHLPNLNEEQRNAFIQSLKDDPSQSANLLAEAKKLNDAQAPKVDNKFNKEIQNAFYVILHLPNLNEEQRNAFIQSLKDDPSQSANLLAEAKKLNDAQAPKVDNKFNKEIQNAFYVILHLPNLNEEQRNAFIQSLKDDPSQSANLLAEAKKLNDAQAPK

SEQ ID NO: 94 - protein, 232 aa, synthetic construct
VDNKFNKEIQNAFYIILHLPNLNEEQRNAFIQSLKDDPSQSANLLAEAKKLNDAQAPKVDNKFNKEIQNAFYIILHLPNLNEEQRNAFIQSLKDDPSQSANLLAEAKKLNDAQAPKVDNKFNKEIQNAFYIILHLPNLNEEQRNAFIQSLKDDPSQSANLLAEAKKLNDAQAPKVDNKFNKEIQNAFYIILHLPNLNEEQRNAFIQSLKDDPSQSANLLAEAKKLNDAQAPK

SEQ ID NO: 95 - protein, 232 aa, synthetic construct
VDLKFLKEIQNAFYLILHLPNLNEEQRNAFIQSLKDDPSQSANLLAEAKKLNDAQAPKVDLKFLKEIQNAFYLILHLPNLNEEQRNAFIQSLKDDPSQSANLLAEAKKLNDAQAPKVDLKFLKEIQNAFYLILHLPNLNEEQRNAFIQSLKDDPSQSANLLAEAKKLNDAQAPKVDLKFLKEIQNAFYLILHLPNLNEEQRNAFIQSLKDDPSQSANLLAEAKKLNDAQAPK

SEQ ID NO: 96 - protein, 232 aa, synthetic construct
VDYKFEKEIQNAFYIILHLPNLNEEQRNAFIQSLKDDPSQSANLLAEAKKLNDAQAPKVDYKFEKEIQNAFYIILHLPNLNEEQRNAFIQSLKDDPSQSANLLAEAKKLNDAQAPKVDYKFEKEIQNAFYIILHLPNLNEEQRNAFIQSLKDDPSQSANLLAEAKKLNDAQAPKVDYKFEKEIQNAFYIILHLPNLNEEQRNAFIQSLKDDPSQSANLLAEAKKLNDAQAPK

SEQ ID NO: 97 - protein, 232 aa, synthetic construct
VDVKFEKEIQNAFYLILHLPNLNEEQRNAFIQSLKDDPSQSANLLAEAKKLNDAQAPKVDVKFEKEIQNAFYLILHLPNLNEEQRNAFIQSLKDDPSQSANLLAEAKKLNDAQAPKVDVKFEKEIQNAFYLILHLPNLNEEQRNAFIQSLKDDPSQSANLLAEAKKLNDAQAPKVDVKFEKEIQNAFYLILHLPNLNEEQRNAFIQSLKDDPSQSANLLAEAKKLNDAQAPK

SEQ ID NO: 98 - protein, 232 aa, synthetic construct
VDLKFNKEIQNAFYLILHLPNLVEEQRNAFIQSLKDDPSQSANLLAEAKKLNDAQAPKVDLKFNKEIQNAFYLILHLPNLVEEQRNAFIQSLKDDPSQSANLLAEAKKLNDAQAPKVDLKFNKEIQNAFYLILHLPNLVEEQRNAFIQSLKDDPSQSANLLAEAKKLNDAQAPKVDLKFNKEIQNAFYLILHLPNLVEEQRNAFIQSLKDDPSQSANLLAEAKKLNDAQAPK

SEQ ID NO: 99 - protein, 232 aa, synthetic construct
VDNKFLKEFQNAFYIILHLPNLVEEQRNAFIQSLKDDPSQSANLLAEAKKLNDAQAPKVDNKFLKEFQNAFYIILHLPNLVEEQRNAFIQSLKDDPSQSANLLAEAKKLNDAQAPKVDNKFLKEFQNAFYIILHLPNLVEEQRNAFIQSLKDDPSQSANLLAEAKKLNDAQAPKVDNKFLKEFQNAFYIILHLPNLVEEQRNAFIQSLKDDPSQSANLLAEAKKLNDAQAPK

SEQ ID NO: 100 - protein, 232 aa, synthetic construct
VDLKFLKEIQNAFYLILHLPNLVEEQRNAFIQSLKDDPSQSANLLAEAKKLNDAQAPKVDLKFLKEIQNAFYLILHLPNLVEEQRNAFIQSLKDDPSQSANLLAEAKKLNDAQAPKVDLKFLKEIQNAFYLILHLPNLVEEQRNAFIQSLKDDPSQSANLLAEAKKLNDAQAPKVDLKFLKEIQNAFYLILHLPNLVEEQRNAFIQSLKDDPSQSANLLAEAKKLNDAQAPK

SEQ ID NO: 101 - protein, 232 aa, synthetic construct
VDLKFEKEIQNAFYIILHLPNLIEEQRNAFIQSLKDDPSQSANLLAEAKKLNDAQAPKVDLKFEKEIQNAFYIILHLPNLIEEQRNAFIQSLKDDPSQSANLLAEAKKLNDAQAPKVDLKFEKEIQNAFYIILHLPNLIEEQRNAFIQSLKDDPSQSANLLAEAKKLNDAQAPKVDLKFEKEIQNAFYIILHLPNLIEEQRNAFIQSLKDDPSQSANLLAEAKKLNDAQAPK

SEQ ID NO: 102 - protein, 232 aa, synthetic construct
VDVKFLKEFQNAFYVILHLPNLYEEQRNAFIQSLKDDPSQSANLLAEAKKLNDAQAPKVDVKFLKEFQNAFYVILHLPNLYEEQRNAFIQSLKDDPSQSANLLAEAKKLNDAQAPKVDVKFLKEFQNAFYVILHLPNLYEEQRNAFIQSLKDDPSQSANLLAEAKKLNDAQAPKVDVKFLKEFQNAFYVILHLPNLYEEQRNAFIQSLKDDPSQSANLLAEAKKLNDAQAPK

SEQ ID NO: 103 - protein, 232 aa, synthetic construct
VDVKFEKEIQNAFYIILHLPNLYEEQRNAFIQSLKDDPSQSANLLAEAKKLNDAQAPKVDVKFEKEIQNAFYIILHLPNLYEEQRNAFIQSLKDDPSQSANLLAEAKKLNDAQAPKVDVKFEKEIQNAFYIILHLPNLYEEQRNAFIQSLKDDPSQSANLLAEAKKLNDAQAPKVDVKFEKEIQNAFYIILHLPNLYEEQRNAFIQSLKDDPSQSANLLAEAKKLNDAQAPK

SEQ ID NO: 104 - protein, 232 aa, synthetic construct
VDLKFLKEFQNAFYIILHLPNLVEEQRNAFIQSLKDDPSQSANLLAEAKKLNDAQAPKVDLKFLKEFQNAFYIILHLPNLVEEQRNAFIQSLKDDPSQSANLLAEAKKLNDAQAPKVDLKFLKEFQNAFYIILHLPNLVEEQRNAFIQSLKDDPSQSANLLAEAKKLNDAQAPKVDLKFLKEFQNAFYIILHLPNLVEEQRNAFIQSLKDDPSQSANLLAEAKKLNDAQAPK

SEQ ID NO: 105 - protein, 232 aa, synthetic construct
VDLKFEKEFQNAFYLILHLPNLIEEQRNAFIQSLKDDPSQSANLLAEAKKLNDAQAPKVDLKFEKEFQNAFYLILHLPNLIEEQRNAFIQSLKDDPSQSANLLAEAKKLNDAQAPKVDLKFEKEFQNAFYLILHLPNLIEEQRNAFIQSLKDDPSQSANLLAEAKKLNDAQAPKVDLKFEKEFQNAFYLILHLPNLIEEQRNAFIQSLKDDPSQSANLLAEAKKLNDAQAPK

SEQ ID NO: 106 - protein, 232 aa, synthetic construct
VDYKFEKEIQNAFYLILHLPNLYEEQRNAFIQSLKDDPSQSANLLAEAKKLNDAQAPKVDYKFEKEIQNAFYLILHLPNLYEEQRNAFIQSLKDDPSQSANLLAEAKKLNDAQAPKVDYKFEKEIQNAFYLILHLPNLYEEQRNAFIQSLKDDPSQSANLLAEAKKLNDAQAPKVDYKFEKEIQNAFYLILHLPNLYEEQRNAFIQSLKDDPSQSANLLAEAKKLNDAQAPK

SEQ ID NO: 107 - protein, 348 aa, synthetic construct
VDLKFEKEIQNAFYIILHLPNLIEEQRNAFIQSLKDDPSQSANLLAEAKKLNDAQAPKVDLKFEKEIQNAFYIILHLPNLIEEQRNAFIQSLKDDPSQSANLLAEAKKLNDAQAPKVDLKFEKEIQNAFYIILHLPNLIEEQRNAFIQSLKDDPSQSANLLAEAKKLNDAQAPKVDLKFEKEIQNAFYIILHLPNLIEEQRNAFIQSLKDDPSQSANLLAEAKKLNDAQAPKVDLKFEKEIQNAFYIILHLPNLIEEQRNAFIQSLKDDPSQSANLLAEAKKLNDAQAPKVDLKFEKEIQNAFYIILHLPNLIEEQRNAFIQSLKDDPSQSANLLAEAKKLNDAQAPK

SEQ ID NO: 108 - protein, 348 aa, synthetic construct
VDVKFLKEIQNAFYVILHLPNLYEEQRNAFIQSLKDDPSQSANLLAEAKKLNDAQAPKVDVKFLKEIQNAFYVILHLPNLYEEQRNAFIQSLKDDPSQSANLLAEAKKLNDAQAPKVDVKFLKEIQNAFYVILHLPNLYEEQRNAFIQSLKDDPSQSANLLAEAKKLNDAQAPKVDVKFLKEIQNAFYVILHLPNLYEEQRNAFIQSLKDDPSQSANLLAEAKKLNDAQAPKVDVKFLKEIQNAFYVILHLPNLYEEQRNAFIQSLKDDPSQSANLLAEAKKLNDAQAPKVDVKFLKEIQNAFYVILHLPNLYEEQRNAFIQSLKDDPSQSANLLAEAKKLNDAQAPK

SEQ ID NO: 109 - protein, 348 aa, synthetic construct
VDLKFLKEFQNAFYIILHLPNLVEEQRNAFIQSLKDDPSQSANLLAEAKKLNDAQAPKVDLKFLKEFQNAFYIILHLPNLVEEQRNAFIQSLKDDPSQSANLLAEAKKLNDAQAPKVDLKFLKEFQNAFYIILHLPNLVEEQRNAFIQSLKDDPSQSANLLAEAKKLNDAQAPKVDLKFLKEFQNAFYIILHLPNLVEEQRNAFIQSLKDDPSQSANLLAEAKKLNDAQAPKVDLKFLKEFQNAFYIILHLPNLVEEQRNAFIQSLKDDPSQSANLLAEAKKLNDAQAPKVDLKFLKEFQNAFYIILHLPNLVEEQRNAFIQSLKDDPSQSANLLAEAKKLNDAQAPK

SEQ ID NO: 110 - protein, 232 aa, synthetic construct
ADNKFNKEQQNAFYEILHLPNLNEEQRNGFIQSLKDDPSQSANLLAEAKKLNDAQAPKADNKFNKEQQNAFYEILHLPNLNEEQRNGFIQSLKDDPSQSANLLAEAKKLNDAQAPKADNKFNKEQQNAFYEILHLPNLNEEQRNGFIQSLKDDPSQSANLLAEAKKLNDAQAPKADNKFNKEQQNAFYEILHLPNLNEEQRNGFIQSLKDDPSQSANLLAEAKKLNDAQAPK

SEQ ID NO: 111 - protein, 232 aa, synthetic construct
ADVKFNKEQQNAFYEILHLPNLNEEQRNGFIQSLKDDPSQSANLLAEAKKLNDAQAPKADVKFNKEQQNAFYEILHLPNLNEEQRNGFIQSLKDDPSQSANLLAEAKKLNDAQAPKADVKFNKEQQNAFYEILHLPNLNEEQRNGFIQSLKDDPSQSANLLAEAKKLNDAQAPKADVKFNKEQQNAFYEILHLPNLNEEQRNGFIQSLKDDPSQSANLLAEAKKLNDAQAPK

SEQ ID NO: 112 - protein, 232 aa, synthetic construct
ADNKFEKEQQNAFYEILHLPNLNEEQRNGFIQSLKDDPSQSANLLAEAKKLNDAQAPKADNKFEKEQQNAFYEILHLPNLNEEQRNGFIQSLKDDPSQSANLLAEAKKLNDAQAPKADNKFEKEQQNAFYEILHLPNLNEEQRNGFIQSLKDDPSQSANLLAEAKKLNDAQAPKADNKFEKEQQNAFYEILHLPNLNEEQRNGFIQSLKDDPSQSANLLAEAKKLNDAQAPK

SEQ ID NO: 113 - protein, 232 aa, synthetic construct
ADNKFNKEIQNAFYEILHLPNLNEEQRNGFIQSLKDDPSQSANLLAEAKKLNDAQAPKADNKFNKEIQNAFYEILHLPNLNEEQRNGFIQSLKDDPSQSANLLAEAKKLNDAQAPKADNKFNKEIQNAFYEILHLPNLNEEQRNGFIQSLKDDPSQSANLLAEAKKLNDAQAPKADNKFNKEIQNAFYEILHLPNLNEEQRNGFIQSLKDDPSQSANLLAEAKKLNDAQAPK

SEQ ID NO: 114 - protein, 232 aa, synthetic construct
ADNKFNKEFQNAFYEILHLPNLNEEQRNGFIQSLKDDPSQSANLLAEAKKLNDAQAPKADNKFNKEFQNAFYEILHLPNLNEEQRNGFIQSLKDDPSQSANLLAEAKKLNDAQAPKADNKFNKEFQNAFYEILHLPNLNEEQRNGFIQSLKDDPSQSANLLAEAKKLNDAQAPKADNKFNKEFQNAFYEILHLPNLNEEQRNGFIQSLKDDPSQSANLLAEAKKLNDAQAPK

SEQ ID NO: 115 - protein, 232 aa, synthetic construct
ADNKFNKEQQNAFYLILHLPNLNEEQRNGFIQSLKDDPSQSANLLAEAKKLNDAQAPKADNKFNKEQQNAFYLILHLPNLNEEQRNGFIQSLKDDPSQSANLLAEAKKLNDAQAPKADNKFNKEQQNAFYLILHLPNLNEEQRNGFIQSLKDDPSQSANLLAEAKKLNDAQAPKADNKFNKEQQNAFYLILHLPNLNEEQRNGFIQSLKDDPSQSANLLAEAKKLNDAQAPK

SEQ ID NO: 116 - protein, 232 aa, synthetic construct
ADNKFNKEQQNAFYIILHLPNLNEEQRNGFIQSLKDDPSQSANLLAEAKKLNDAQAPKADNKFNKEQQNAFYIILHLPNLNEEQRNGFIQSLKDDPSQSANLLAEAKKLNDAQAPKADNKFNKEQQNAFYIILHLPNLNEEQRNGFIQSLKDDPSQSANLLAEAKKLNDAQAPKADNKFNKEQQNAFYIILHLPNLNEEQRNGFIQSLKDDPSQSANLLAEAKKLNDAQAPK

SEQ ID NO: 117 - protein, 232 aa, synthetic construct
ADVKFEKEIQNAFYLILHLPNLNEEQRNGFIQSLKDDPSQSANLLAEAKKLNDAQAPKADVKFEKEIQNAFYLILHLPNLNEEQRNGFIQSLKDDPSQSANLLAEAKKLNDAQAPKADVKFEKEIQNAFYLILHLPNLNEEQRNGFIQSLKDDPSQSANLLAEAKKLNDAQAPKADVKFEKEIQNAFYLILHLPNLNEEQRNGFIQSLKDDPSQSANLLAEAKKLNDAQAPK

SEQ ID NO: 118 - protein, 58 aa, synthetic construct
ADVKFNKEQQNAFYEILHLPNLNEEQRNGFIQSLKDDPSQSANLLAEAKKLNDAQAPK

SEQ ID NO: 119 - protein, 58 aa, synthetic construct
ADNKFEKEQQNAFYEILHLPNLNEEQRNGFIQSLKDDPSQSANLLAEAKKLNDAQAPK

SEQ ID NO: 120 - protein, 58 aa, synthetic construct
ADNKFNKEIQNAFYEILHLPNLNEEQRNGFIQSLKDDPSQSANLLAEAKKLNDAQAPK

SEQ ID NO: 121 - protein, 58 aa, synthetic construct
ADNKFNKEFQNAFYEILHLPNLNEEQRNGFIQSLKDDPSQSANLLAEAKKLNDAQAPK

SEQ ID NO: 122 - protein, 58 aa, synthetic construct
ADNKFNKEQQNAFYLILHLPNLNEEQRNGFIQSLKDDPSQSANLLAEAKKLNDAQAPK

SEQ ID NO: 123 - protein, 58 aa, synthetic construct
ADNKFNKEQQNAFYIILHLPNLNEEQRNGFIQSLKDDPSQSANLLAEAKKLNDAQAPK

SEQ ID NO: 124 - protein, 58 aa, synthetic construct
ADVKFEKEIQNAFYLILHLPNLNEEQRNGFIQSLKDDPSQSANLLAEAKKLNDAQAPK